European Patent Specification EP 3 271 387 B1, published December 6, 2023. Title: Trispecific binding molecules for treating HBV infection and associated conditions. Applicant: Helmholtz Zentrum München - Deutsches Forschungszentrum für Gesundheit und Umwelt (GmbH) et al. The sequence listing filed with the application follows.

SEQUENCE LISTING (51 sequences)

SEQ ID NO: 1 - protein, 8 aa, Artificial Sequence
  CDR1 of scFv C8 heavy chain
GFTFSGYA

SEQ ID NO: 2 - protein, 8 aa, Artificial Sequence
  CDR2 of scFv C8 heavy chain
ISGSGGST

SEQ ID NO: 3 - protein, 21 aa, Artificial Sequence
  CDR3 of scFv C8 heavy chain
AKPPGRQEYYGSSIYYFPLGN

SEQ ID NO: 4 - protein, 6 aa, Artificial Sequence
  CDR1 of scFv C8 light chain
NIGSKS

SEQ ID NO: 5 - protein, 3 aa, Artificial Sequence
  CDR2 of scFv C8 light chain
DDS

SEQ ID NO: 6 - protein, 11 aa, Artificial Sequence
  CDR3 of scFv C8 light chain
QVWDSSSDLVV

SEQ ID NO: 7 - protein, 8 aa, Artificial Sequence
  CDR1 of scFv 5F9 heavy chain
GFTFNNYA

SEQ ID NO: 8 - protein, 8 aa, Artificial Sequence
  CDR2 of scFv 5F9 heavy chain
INSDGRST

SEQ ID NO: 9 - protein, 8 aa, Artificial Sequence
  CDR3 of scFv 5F9 heavy chain
ARTFYADY

SEQ ID NO: 10 - protein, 6 aa, Artificial Sequence
  CDR1 of scFv 5F9 light chain
QNVDTT

SEQ ID NO: 11 - protein, 3 aa, Artificial Sequence
  CDR2 of scFv 5F9 light chain
WAS

SEQ ID NO: 12 - protein, 9 aa, Artificial Sequence
  CDR3 of scFv 5F9 light chain
QQYSIFPYT

SEQ ID NO: 13 - protein, 8 aa, Artificial Sequence
  CDR1 of scFv 5A19 heavy chain
GFTFSSYA

SEQ ID NO: 14 - protein, 8 aa, Artificial Sequence
  CDR2 of scFv 5A19 heavy chain
VSSDGSYA

SEQ ID NO: 15 - protein, 9 aa, Artificial Sequence
  CDR3 of scFv 5A19 heavy chain
ASFNWDVAY

SEQ ID NO: 16 - protein, 12 aa, Artificial Sequence
  CDR1 of scFv 5A19 light chain
QSLLNTRTRKSY

SEQ ID NO: 17 - protein, 3 aa, Artificial Sequence
  CDR2 of scFv 5A19 light chain
WAS

SEQ ID NO: 18 - protein, 8 aa, Artificial Sequence
  CDR3 of scFv 5A19 light chain
KQSYSLYT

SEQ ID NO: 19 - protein, 8 aa, Artificial Sequence
  CDR1 of scFv OKT3 heavy chain
GYTFTRYT

SEQ ID NO: 20 - protein, 8 aa, Artificial Sequence
  CDR2 of scFv OKT3 heavy chain
INPSRGYT

SEQ ID NO: 21 - protein, 12 aa, Artificial Sequence
  CDR3 of scFv OKT3 heavy chain
ARYYDDHYCLDY

SEQ ID NO: 22 - protein, 5 aa, Artificial Sequence
  CDR1 of scFv OKT3 light chain
SSVSY

SEQ ID NO: 23 - protein, 3 aa, Artificial Sequence
  CDR2 of scFv OKT3 light chain
DTS

SEQ ID NO: 24 - protein, 9 aa, Artificial Sequence
  CDR3 of scFv OKT3 light chain
QQWSSNPFT

SEQ ID NO: 25 - protein, 8 aa, Artificial Sequence
  CDR1 of scFv 9.3 heavy chain
GFSLSDYG

SEQ ID NO: 26 - protein, 7 aa, Artificial Sequence
  CDR2 of scFv 9.3 heavy chain
IWAGGGT

SEQ ID NO: 27 - protein, 14 aa, Artificial Sequence
  CDR3 of scFv 9.3 heavy chain
ARDKGYSYYYSMDY

SEQ ID NO: 28 - protein, 10 aa, Artificial Sequence
  CDR1 of scFv 9.3 light chain
ESVEYYVTSL

SEQ ID NO: 29 - protein, 3 aa, Artificial Sequence
  CDR2 of scFv 9.3 light chain
AAS

SEQ ID NO: 30 - protein, 9 aa, Artificial Sequence
  CDR3 of scFv 9.3 light chain
QQSRKVPYT

SEQ ID NO: 31 - protein, 8 aa, Artificial Sequence
  CDR1 of scFv A9 heavy chain
GYTFTNYW

SEQ ID NO: 32 - protein, 8 aa, Artificial Sequence
  CDR2 of scFv A9 heavy chain
IYPGGGYT

SEQ ID NO: 33 - protein, 10 aa, Artificial Sequence
  CDR3 of scFv A9 heavy chain
ARSASWYFDV

SEQ ID NO: 34 - protein, 9 aa, Artificial Sequence
  CDR1 of scFv A9 light chain
TGTVTTSNY

SEQ ID NO: 35 - protein, 3 aa, Artificial Sequence
  CDR2 of scFv A9 light chain
HTN

SEQ ID NO: 36 - protein, 9 aa, Artificial Sequence
  CDR3 of scFv A9 light chain
ALWYNNHWV

SEQ ID NO: 37 - protein, 8 aa, Artificial Sequence
  CDR1 of scFv NCAM29.2 heavy chain
GFTFSSFG

SEQ ID NO: 38 - protein, 8 aa, Artificial Sequence
  CDR2 of scFv NCAM29.2 heavy chain
ISSGSYAI

SEQ ID NO: 39 - protein, 14 aa, Artificial Sequence
  CDR3 of scFv NCAM29.2 heavy chain
VRGRRLGEGYAMDY

SEQ ID NO: 40 - protein, 12 aa, Artificial Sequence
  CDR1 of scFv NCAM29.2 light chain
QSLLYSSNQKNY

SEQ ID NO: 41 - protein, 3 aa, Artificial Sequence
  CDR2 of scFv NCAM29.2 light chain
WAS

SEQ ID NO: 42 - protein, 7 aa, Artificial Sequence
  CDR3 of scFv NCAM29.2 light chain
QQYSSWT

SEQ ID NO: 43 - protein, 794 aa, Artificial Sequence
  Anti-HBsAg scFv [C8]^Glycin-Serin-Linker^hIgG1-Fc[C245S,L259F,L26 0E,G262A,A355T]^StrepTag^Glycin-Linker^anti-CD3 scFv [OKT3]
MDFEVQIFSFLLISASVIMSRMAEVQLVESGGGLLQPGGSLRLSCAASGFTFSGYAMSWVRQAPGKGLEWVSSISGSGGSTYYADSVKGRFTISRDNSKNTLYLQMNSLRAEDTALYYCAKPPGRQEYYGSSIYYFPLGNWGQGTLVTVSSASTKGPKLEEGEFSEARVQSALTQPASVSVAPGQTARITCGGNNIGSKSVHWYQQKPGQAPVLVVYDDSDRPSGIPERFSGSNSGNTATLTISRVEAGDEADYYCQVWDSSSDLVVFGGGTKLTVLGNSGGGGSGGGGSGGGGSASEPKSSDKTHTCPPCPAPEFEGAPSVFLFPPKPKDTLMISRTPEVTCVVVDVSHEDPEVKFNWYVDGVEVHNAKTKPREEQYNSTYRVVSVLTVLHQDWLNGKEYKCKVSNKALPTPIEKTISKAKGQPREPQVYTLPPSRDELTKNQVSLTCLVKGFYPSDIAVEWESNGQPENNYKTTPPVLDSDGSFFLYSKLTVDKSRWQQGNVFSCSVMHEALHNHYTQKSLSLSPGKDPGWSHPQFEKSRGGGGQVQLQQSGAELARPGASVKMSCKASGYTFTRYTMHWVKQRPGQGLEWIGYINPSRGYTNYNQKFKDKATLTTDKSSSTAYMQLSSLTSEDSAVYYCARYYDDHYCLDYWGQGTTLTVSSGNSGGGGSGGGGSGGGGSASQIVLTQSPAIMSASPGEKVTMTCSASSSVSYMNWYQQKSGTSPKRWIYDTSKLASGVPAHFRGSGSGTSYSLTISGMEAEDAATYYCQQWSSNPFTFGSGTKLEINGNS

SEQ ID NO: 44 - protein, 793 aa, Artificial Sequence [sequence omitted]

SEQ ID NO: 45 - protein, 792 aa, Artificial Sequence
  Anti-HBsAg scFv [C8]^Glycin-Serin-Linker^hIgG1-Fc[C245S,L259F,L26 0E,G262A,A355T]^StrepTag^Glycin-Linker^ StrepTag^anti-CD16 scFv [A9]
MDFEVQIFSFLLISASVIMSRMAEVQLVESGGGLLQPGGSLRLSCAASGFTFSGYAMSWVRQAPGKGLEWVSSISGSGGSTYYADSVKGRFTISRDNSKNTLYLQMNSLRAEDTALYYCAKPPGRQEYYGSSIYYFPLGNWGQGTLVTVSSASTKGPKLEEGEFSEARVQSALTQPASVSVAPGQTARITCGGNNIGSKSVHWYQQKPGQAPVLVVYDDSDRPSGIPERFSGSNSGNTATLTISRVEAGDEADYYCQVWDSSSDLVVFGGGTKLTVLGNSGGGGSGGGGSGGGGSASEPKSSDKTHTCPPCPAPEFEGAPSVFLFPPKPKDTLMISRTPEVTCVVVDVSHEDPEVKFNWYVDGVEVHNAKTKPREEQYNSTYRVVSVLTVLHQDWLNGKEYKCKVSNKALPTPIEKTISKAKGQPREPQVYTLPPSRDELTKNQVSLTCLVKGFYPSDIAVEWESNGQPENNYKTTPPVLDSDGSFFLYSKLTVDKSRWQQGNVFSCSVMHEALHNHYTQKSLSLSPGKDPGWSHPQFEKSRGGGGQVQLQQSGAELVRPGTSVKISCKASGYTFTNYWLGWVKQRPGHGLEWIGDIYPGGGYTNYNEKFKGKATVTADTSSRTAYVQVRSLTSEDSAVYFCARSASWYFDVWGAGTTVTVSSGNSGGGGSGGGGSGGGGSASQAVVTQESALTTSPGETVTLTCRSNTGTVTTSNYANWVQEKPDHLFTGLIGHTNNRAPGVPARFSGSLIGDKAALTITGAQTEDEAIYFCALWYNNHWVFGGGTKLTVL

SEQ ID NO: 46 - protein, 799 aa, Artificial Sequence [sequence omitted]

SEQ ID NO: 47 - protein, 15 aa, Artificial Sequence
  Linker
GGGGSGGGGSGGGGS

SEQ ID NO: 48 - protein, 17 aa, Artificial Sequence
  Linker
AKTTPKLEEGEFSEARV

SEQ ID NO: 49 - protein, 20 aa, Artificial Sequence
  Linker
GGGGSGGGGSGGGGSGGGGS

SEQ ID NO: 50 - protein, 835 aa, Artificial Sequence
  C8-hIgG1Fcmut-OKT3 with Jun leucine zipper dimerization domain
MDFEVQIFSFLLISASVIMSRMAEVQLVESGGGLLQPGGSLRLSCAASGFTFSGYAMSWVRQAPGKGLEWVSSISGSGGSTYYADSVKGRFTISRDNSKNTLYLQMNSLRAEDTALYYCAKPPGRQEYYGSSIYYFPLGNWGQGTLVTVSSASTKGPKLEEGEFSEARVQSALTQPASVSVAPGQTARITCGGNNIGSKSVHWYQQKPGQAPVLVVYDDSDRPSGIPERFSGSNSGNTATLTISRVEAGDEADYYCQVWDSSSDLVVFGGGTKLTVLGNSGGGGSGGGGSGGGGSASRIARLEEKVKTLKAQNSELASTANMLREQVAQLKQKVMNYSSEPKSSDKTHTCPPCPAPPAAGPSVFLFPPKPKDTLMISRTPEVTCVVVDVSHEDPEVKFNWYVDGVEVHNAKTKPREEQYNSTYRVVSVLTVLHQDWLNGKEYKCAVSNKGLASSIEKTISKAKGQPREPQVYTLPPSRDELTKNQVSLTCLVKGFYPSDIAVEWESNGQPENNYKTTPPVLDSDGSFFLYSKLTVDKSRWQQGNVFSCSVMHEALHNHYTQKSLSLSPGKDPGWSHPQFEKSRGGGGQVQLQQSGAELARPGASVKMSCKASGYTFTRYTMHWVKQRPGQGLEWIGYINPSRGYTNYNQKFKDKATLTTDKSSSTAYMQLSSLTSEDSAVYYCARYYDDHYCLDYWGQGTTLTVSSGNSGGGGSGGGGSGGGGSASQIVLTQSPAIMSASPGEKVTMTCSASSSVSYMNWYQQKSGTSPKRWIYDTSKLASGVPAHFRGSGSGTSYSLTISGMEAEDAATYYCQQWSSNPFTFGSGTKLEINGNS

SEQ ID NO: 51 - protein, 834 aa, Artificial Sequence
  C8- hIgG1Fcmut-9.3 with Fos leucine zipper dimerization domain
MDFEVQIFSFLLISASVIMSRMAEVQLVESGGGLLQPGGSLRLSCAASGFTFSGYAMSWVRQAPGKGLEWVSSISGSGGSTYYADSVKGRFTISRDNSKNTLYLQMNSLRAEDTALYYCAKPPGRQEYYGSSIYYFPLGNWGQGTLVTVSSASTKGPKLEEGEFSEARVQSALTQPASVSVAPGQTARITCGGNNIGSKSVHWYQQKPGQAPVLVVYDDSDRPSGIPERFSGSNSGNTATLTISRVEAGDEADYYCQVWDSSSDLVVFGGGTKLTVLGNSGGGGSGGGGSGGGGSASLTDTLQAETDQLEDKKSALQTEIANLLKEKEKLEFILAAYSSEPKSSDKTHTCPPCPAPPAAGPSVFLFPPKPKDTLMISRTPEVTCVVVDVSHEDPEVKFNWYVDGVEVHNAKTKPREEQYNSTYRVVSVLTVLHQDWLNGKEYKCAVSNKGLASSIEKTISKAKGQPREPQVYTLPPSRDELTKNQVSLTCLVKGFYPSDIAVEWESNGQPENNYKTTPPVLDSDGSFFLYSKLTVDKSRWQQGNVFSCSVMHEALHNHYTQKSLSLSPGKDPGWSHPQFEKSSGGGGQVQLQESGPGLVTPSQSLSITCTVSGFSLSDYGVHWVRQSPGQGLEWLGVIWAGGGTNYNSALMSRKSISKDNSKSQVFLKMNSLQADDTAVYYCARDKGYSYYYSMDYWGQGTTVTVSSRGGGSGGGGSGGGGSDIELTQSPASLAVSLGQRATISCRASESVEYYVTSLMQWYQQKPGQPPKLLIFAASNVESGVPARFSGSGSGTNFSLNIHPVDEDDVAMYFCQQSRKVPYTFGGGTKLEIKR